European Patent Application EP 4 755 898 A1, published June 10, 2026. Title: A method of synthesizing oligonucleotide. Applicant: 日東電工株式会社. Application JP. The sequence listing filed with the application follows.

SEQUENCE LISTING (8 sequences)

SEQ ID NO: 1 - DNA, 24 bp, synthetic construct
  source 1..24: mol_type = other DNA
  modified_base 1..24: mod_base = OTHER; note = phosphorothioate bond
tcgacgtattgacgtattgacgta

SEQ ID NO: 2 - DNA, 24 bp, synthetic construct
  source 1..24: mol_type = other DNA
tcgacgtattgacgtattgacgta

SEQ ID NO: 3 - DNA, 24 bp, synthetic construct
  source 1..24: mol_type = other DNA
  modified_base 1..24: mod_base = OTHER; note = phosphorothioate bond
cgtacgtacgtacgtacgtacgta

SEQ ID NO: 4 - DNA, 21 bp, synthetic construct
  source 1..21: mol_type = other DNA
  modified_base 1..21: mod_base = OTHER; note = phosphorothioate bond
tataccgattaagcgaagttt

SEQ ID NO: 5 - DNA, 25 bp, synthetic construct
  source 1..25: mol_type = other DNA
  modified_base 1..25: mod_base = OTHER; note = phosphorothioate bond
tttgaagcgaattagccatatcgta

SEQ ID NO: 6 - RNA, 23 nt, synthetic construct
  source 1..23: mol_type = other RNA
  modified_base 1..23: mod_base = OTHER; note = phosphorothioate bond
  modified_base 1: mod_base = gm
  modified_base 2: mod_base = gm
  modified_base 3: mod_base = um
  modified_base 4: mod_base = um
  modified_base 5: mod_base = um
  modified_base 6: mod_base = OTHER; note = 2'-O-methyladenosine
  modified_base 7: mod_base = OTHER; note = 2'-O-methyladenosine
  modified_base 8: mod_base = cm
  modified_base 9: mod_base = gm
  modified_base 10: mod_base = um
  modified_base 11: mod_base = OTHER; note = 2'-O-methyladenosine
  modified_base 12: mod_base = cm
  modified_base 13: mod_base = gm
  modified_base 14: mod_base = um
  modified_base 15: mod_base = OTHER; note = 2'-O-methyladenosine
  modified_base 16: mod_base = cm
  modified_base 17: mod_base = gm
  modified_base 18: mod_base = um
  modified_base 19: mod_base = OTHER; note = 2'-O-methyladenosine
  modified_base 20: mod_base = cm
  modified_base 21: mod_base = gm
  modified_base 22: mod_base = um
  modified_base 23: mod_base = OTHER; note = 2'-O-methyladenosine
ggtttaacgtacgtacgtacgta

SEQ ID NO: 7 - DNA, 24 bp, synthetic construct
  source 1..24: mol_type = other DNA
  modified_base 7..24: mod_base = OTHER; note = phosphorothioate bond
tcgacgtattgacgtattgacgta

SEQ ID NO: 8 - DNA, 24 bp, synthetic construct
  source 1..24: mol_type = other DNA
  modified_base 4..22: mod_base = OTHER; note = phosphorothioate bond
tcgacgtattgacgtattgacgta